European Patent Application EP 4 537 815 A1, published April 16, 2025. Title: Composition comprising a lasso peptide formulated in a pharmaceutically acceptable nanoemulsion. Applicant: Muséum National d'Histoire Naturelle. Application EP 22306978.2, filed January 16, 2023. The sequence listing filed with the application follows.

SEQUENCE LISTING (7 sequences)

SEQ ID NO: 1 - protein, 21 aa, Streptomyces
CLGVGSCNDFAGCGYAIVCFW

SEQ ID NO: 2 - protein, 20 aa, Streptomyces sviceus
CVWGGDCTDFLGCGTAWICV

SEQ ID NO: 3 - protein, 20 aa, Streptomyces
CLPSGDCPDFLGCGRAIWCI

SEQ ID NO: 4 - protein, 21 aa, Streptomyces
CLGIGSCNDFAGCGYAIVCFW

SEQ ID NO: 5 - protein, 21 aa, Streptomyces
CLGIGSCNDFAGCGYAVVCFW

SEQ ID NO: 6 - protein, 21 aa, Streptomyces specialis
CLGVGSCVDFAGCGYAVVCFW

SEQ ID NO: 7 - protein, 21 aa, Streptomyces humidus
CLGIGSCDDFAGCGYAIVCFW